European Patent Application EP 4 144 349 A1, published March 8, 2023. Title: NUCLEIC ACIDS INDUCING RNA INTERFERENCE INCLUDING 8-OXOGUANINE, MICRO RNA INCLUDING 8-OXOGUANINE, AND USE THEREOF. Applicant: Korea University Research and Business Foundation. The sequence listing filed with the application follows.

SEQUENCE LISTING (70 sequences)

SEQ ID NO: 1 - RNA, 22 nt, Artificial Sequence
  miR-1:2(8-oxoguanine)
  misc_difference (2): 8-oxoguanine
uggaauguaaagaaguauguau

SEQ ID NO: 2 - RNA, 22 nt, Artificial Sequence
  miR-1:3(8-oxoguanine)
  misc_difference (3): 8-oxoguanine
uggaauguaaagaaguauguau

SEQ ID NO: 3 - RNA, 22 nt, Artificial Sequence
  miR-1:7(8-oxoguanine)
  misc_difference (7): 8-oxoguanine
uggaauguaaagaaguauguau

SEQ ID NO: 4 - RNA, 7 nt, Artificial Sequence
  miR-1 2oxo site
acauuca

SEQ ID NO: 5 - RNA, 7 nt, Artificial Sequence
  miR-1 3oxo site
acauuac

SEQ ID NO: 6 - RNA, 7 nt, Artificial Sequence
  miR-1 7oxo site
aaauucc

SEQ ID NO: 7 - RNA, 22 nt, Artificial Sequence
  miR-1
  gene (1)..(22): miR-1
uggaauguaaagaaguauguau

SEQ ID NO: 8 - RNA, 23 nt, Artificial Sequence
  miR-1 passenger
acauacuucuuuauaugcccaua

SEQ ID NO: 9 - RNA, 22 nt, Artificial Sequence
  miR-1:2GU
uugaauguaaagaaguauguau

SEQ ID NO: 10 - RNA, 22 nt, Artificial Sequence
  miR-1:3GU
uguaauguaaagaaguauguau

SEQ ID NO: 11 - RNA, 22 nt, Artificial Sequence
  miR-1:7GU
uggaauuuaaagaaguauguau

SEQ ID NO: 12 - RNA, 22 nt, Artificial Sequence
  cel-miR-67
  gene (1)..(22): cel-miR-67
ucacaaccuccuagaaagagua

SEQ ID NO: 13 - RNA, 24 nt, Artificial Sequence
  thymidine deoxynucleotide (dT)
  misc_difference (23)..(24): thymidine deoxynucleotide (dT)
ucacaaccuccuagaaagaguatt

SEQ ID NO: 14 - RNA, 24 nt, Artificial Sequence
  passenger strand
  misc_difference (23)..(24): thymidine deoxynucleotide (dT)
uacucuuucuaggagguugugatt

SEQ ID NO: 15 - RNA, 80 nt, Artificial Sequence
  39-oxo-R
  misc_difference (22): 8-oxoguanine
ccuggucccagacuaaagaaugcuugacaguuaucucguaugccgucuucucgagguagcggaaccgugagcuuugaagu

SEQ ID NO: 16 - RNA, 80 nt, Artificial Sequence; identical to SEQ ID NO: 15
  39R

SEQ ID NO: 17 - RNA, 22 nt, Artificial Sequence
  8-oxoguanine spike-in
  misc_difference (2)..(3): 8-oxoguanine
uggaauguaaagaaguauguau

SEQ ID NO: 18 - RNA, 22 nt, Artificial Sequence
  G spike-in
uggaauguaaagaaguauguau

SEQ ID NO: 19 - RNA, 22 nt, Artificial Sequence
  miRNA:8-oxoguanine spike-in
  misc_difference (5): 8-oxoguanine
uaaggcacgcggugaaugccaa

SEQ ID NO: 20 - RNA, 7 nt, Artificial Sequence
  miR-1 seed site
acauucc

SEQ ID NO: 21 - RNA, 7 nt, Artificial Sequence
  cont NT site
gguugug

SEQ ID NO: 22 - DNA, 46 bp, Artificial Sequence
  oligo dT adaptor primer
gcgagcacagaattaatacgactcactataggttttttttttttvn

SEQ ID NO: 23 - DNA, 26 bp, Artificial Sequence
  miRNA reverse primer
gcgagcacagaattaatacgactcac

SEQ ID NO: 24 - DNA, 22 bp, Artificial Sequence
  8-oxoguanine or G spike-in forward primer
tggaatgtaaagaagtatgtat

SEQ ID NO: 25 - DNA, 26 bp, Artificial Sequence
  8-oxoguanine or G spike-in reverse primer
gcgagcacagaattaatacgactcac

SEQ ID NO: 26 - DNA, 22 bp, Artificial Sequence
  miRNA:8-oxoguanine spike-in forward primer
taaggcacgcggtgaatgccaa

SEQ ID NO: 27 - DNA, 26 bp, Artificial Sequence
  miRNA:8-oxoguanine spike-in reverse primer
gcgagcacagaattaatacgactcac

SEQ ID NO: 28 - DNA, 20 bp, Artificial Sequence
  control forward primer
cgcttcggcagcacatatac

SEQ ID NO: 29 - DNA, 20 bp, Artificial Sequence
  control reverse primer
ttcacgaatttgcgtgtcat

SEQ ID NO: 30 - DNA, 45 bp, Artificial Sequence
  RT primer
acttcaaagctcacggttccgctacctcgagaagacggcatacga

SEQ ID NO: 31 - DNA, 21 bp, Artificial Sequence
  39-oxo-R or 39R forward primer
cctggtcccagactaaagaat

SEQ ID NO: 32 - DNA, 21 bp, Artificial Sequence
  39-oxo-R or 39R reverse primer
acttcaaagctcacggttccg

SEQ ID NO: 33 - RNA, 22 nt, Artificial Sequence
  22nt synthetic RNA
  misc_difference (7): 8-oxoguanine
uggaauguaaagaaguauguau

SEQ ID NO: 34 - RNA, 22 nt, Artificial Sequence
  3'adaptor : 5'-adenylation
  misc_difference (2): methyl-phosphonate guanine
  misc_difference (2): dideoxy-cytosine
tggaattctcgggtgccaaggc

SEQ ID NO: 35 - RNA, 31 nt, Artificial Sequence
  5'adaptor
  misc_difference (31): 2'-methoxy-C
guucagaguucuacaguccgacgaucnnnnc

SEQ ID NO: 36 - DNA, 22 bp, Artificial Sequence
  RT primer
gccttggcacccgagaattcca

SEQ ID NO: 37 - DNA, 50 bp, Artificial Sequence
  universal forward primer
aatgatacggcgaccaccgagatctacacgttcagagttctacagtccga

SEQ ID NO: 38 - DNA, 57 bp, Artificial Sequence
  barcode primer
caagcagaagacggcatacgagatgtgactggagttccttggcacccgagaattcca

SEQ ID NO: 39 - DNA, 42 bp, Artificial Sequence
  miR-1-seed site forward primer
tcgagacattccacattccacattccacattccacattccgc

SEQ ID NO: 40 - DNA, 42 bp, Artificial Sequence
  miR-1-seed site reverse primer
ggccgcggaatgtggaatgtggaatgtggaatgtggaatgtc

SEQ ID NO: 41 - DNA, 42 bp, Artificial Sequence
  miR-1-2oxo site forward primer
tcgagacattcaacattcaacattcaacattcaacattcagc

SEQ ID NO: 42 - DNA, 42 bp, Artificial Sequence
  miR-1-2oxo site reverse primer
ggccgctgaatgttgaatgttgaatgttgaatgttgaatgtc

SEQ ID NO: 43 - DNA, 42 bp, Artificial Sequence
  miR-1-3oxo site forward primer
tcgagacattacacattacacattacacattacacattacgc

SEQ ID NO: 44 - DNA, 42 bp, Artificial Sequence
  miR-1-3oxo site reverse primer
ggccgcgtaatgtgtaatgtgtaatgtgtaatgtgtaatgtc

SEQ ID NO: 45 - DNA, 42 bp, Artificial Sequence
  miR-1-7oxo site forward primer
tcgagaaattccaaattccaaattccaaattccaaattccgc

SEQ ID NO: 46 - DNA, 42 bp, Artificial Sequence
  miR-1-7oxo site reverse primer
ggccgcggaatttggaatttggaatttggaatttggaatttc

SEQ ID NO: 47 - DNA, 42 bp, Artificial Sequence
  miR-1 control site forward primer
tcgagactttccactttccactttccactttccactttccgc

SEQ ID NO: 48 - DNA, 42 bp, Artificial Sequence
  miR-1 control site reverse primer
ggccgcggaaagtggaaagtggaaagtggaaagtggaaagtc

SEQ ID NO: 49 - DNA, 30 bp, Artificial Sequence
  NheI and XhoI site forward primer
taggctagccaccatggtgagcaagggcga

SEQ ID NO: 50 - DNA, 45 bp, Artificial Sequence
  NheI and XhoI site reverse primer
gggctcgagcgatcgcctagaattacttgtacagctcgtccatgc

SEQ ID NO: 51 - DNA, 32 bp, Artificial Sequence
  ApaI and XbaI site forward primer
gaagggccctatgagcgagctgatcaaggaga

SEQ ID NO: 52 - DNA, 36 bp, Artificial Sequence
  ApaI and XbaI site reverse primer
gactctagaattattatctgtgccccagtttgctag

SEQ ID NO: 53 - DNA, 36 bp, Artificial Sequence
  residual 33bp of hluc+ sequences forward primer
gtactgttggtaaagccaccatgagcgagctgatca

SEQ ID NO: 54 - DNA, 36 bp, Artificial Sequence
  residual 33bp of hluc+ sequences reverse primer
tccttgatcagctcgctcatggtggctttaccaaca

SEQ ID NO: 55 - DNA, 22 bp, Artificial Sequence
  hGH poly (A) forward primer
ccaccagccttgtcctaataaa

SEQ ID NO: 56 - DNA, 19 bp, Artificial Sequence
  hGH poly (A) reverse primer
cagcttggttcccaataga

SEQ ID NO: 57 - DNA, 122 bp, Artificial Sequence
  anti-7oxo (alpha-MHC 13x) forward primer
tcgacaaattccaaaaattccataaattccagaaattccacaaattccaaaaattccacaaattccataaattccagaaattccaaaaattccataaattccagaaattccacaaattccaa

SEQ ID NO: 58 - DNA, 122 bp, Artificial Sequence
  anti-7oxo (alpha-MHC 13x) reverse primer
agctttggaatttgtggaatttctggaatttatggaatttttggaatttctggaatttatggaatttgtggaatttttggaatttgtggaatttctggaatttatggaatttttggaatttg

SEQ ID NO: 59 - DNA, 122 bp, Artificial Sequence
  cont (anti-NT 13x) forward primer
tcgacggttgtgaaggttgtgatggttgtgagggttgtgacggttgtgaaggttgtgacggttgtgatggttgtgagggttgtgaaggttgtgatggttgtgagggttgtgacggttgtgaa

SEQ ID NO: 60 - DNA, 122 bp, Artificial Sequence
  cont (anti-NT 13x) reverse primer
agctttcacaaccgtcacaaccctcacaaccatcacaaccttcacaaccctcacaaccatcacaaccgtcacaaccttcacaaccgtcacaaccctcacaaccatcacaaccttcacaaccg

SEQ ID NO: 61 - DNA, 35 bp, Artificial Sequence
  hGH poly (A) forward primer
taaattccaaattccagaaattccacaaattccat

SEQ ID NO: 62 - DNA, 20 bp, Artificial Sequence
  hGH poly (A) reverse primer
ccagcttggttcccaataga

SEQ ID NO: 63 - DNA, 35 bp, Artificial Sequence; identical to SEQ ID NO: 61
  anti-7oxo (4x) primer

SEQ ID NO: 64 - RNA, 20 nt, Artificial Sequence
  8-oxo deoxyguanosine RNA spike-in
  misc_difference (5): 8-oxo deoxyguanosine
uaaggcacgcggugaaugcc

SEQ ID NO: 65 - RNA, 23 nt, Artificial Sequence
  miR-122:2,3(8-oxoguanine)
  misc_difference (2): 8-oxoguanine
  misc_difference (3): 8-oxoguanine
ugggagugugacaaugguguuug

SEQ ID NO: 66 - RNA, 19 nt, Artificial Sequence
  let-7:4(8-oxoguanine)
  misc_difference (4): 8-oxoguanine
ugaguaguagguuguauag

SEQ ID NO: 67 - RNA, 19 nt, Artificial Sequence
  miR-124:4(8-oxoguanine)
  misc_difference (4): 8-oxoguanine
uaaggcacgcggugaaugc

SEQ ID NO: 68 - RNA, 22 nt, Artificial Sequence
  miR-122
uggagugugacaaugguguuug

SEQ ID NO: 69 - RNA, 19 nt, Artificial Sequence
  let-7
ugaguaguagguuguauag

SEQ ID NO: 70 - RNA, 19 nt, Artificial Sequence
  miR-124
uaaggcacgcggugaaugc